European Patent Application EP 4 703 377 A1, published March 4, 2026. Title: Anti-Influenza Virus Antibody. Applicant: JAPAN as represented by DIRECTOR GENERAL of National Institute of Infectious Diseases. The sequence listing filed with the application follows.

SEQUENCE LISTING (98 sequences)

SEQ ID NO: 1 - protein, 151 aa, Alphainfluenzavirus influenzae
YHHQNEQGSGYAADLKSTQNAIDEITNKVNSVIEKMNTQFTAVGKEFNHLEKRIENLNKKVDDGFLDIWTYNAELLVLLENERTLDYHDSNVKNLYEKVRSQLKNNAKEIGNGCFEFYHKCDNTCMESVKNGTYDYPKYSEEAKLNREEID

SEQ ID NO: 2 - protein, 151 aa, Alphainfluenzavirus influenzae
YHHSNDQGSGYAADKESTQKAFNGITNKVNSVIEKMNTQFEAVGKEFSNLEKRLENLNKKMEDGFLDVWTYNAELLVLMENERTLDFHDSNVKNLYDKVRMQLRDNVKELGNGCFEFYHKCDNECMDSVKNGTYDYPKYEEESKLNRNEIK

SEQ ID NO: 3 - protein, 151 aa, Alphainfluenzavirus influenzae
FRHQNSEGTGQAADLKSTQAAIDQINGKLNRVIEKTNEKFHQIEKEFSEVEGRIQDLEKYVEDTKIDLWSYNAELLVALENQHTIDLTDSEMNKLFEKTRRQLRENAEDMGNGCFKIYHKCDNACIESIRNGTYDHDVYRDEALNNRFQIK

SEQ ID NO: 4 - protein, 151 aa, Alphainfluenzavirus influenzae
FRHQNAEGTGTAADLKSTQAAIDQINGKLNRLIEKTNEKYHQIEKEFEQVEGRIQDLEKYVEDTKIDLWSYNAEFLVALENQHTIDVTDSEMNKLFERVRRQLRENAEDKGNGCFEIFHQCDNNCIESIRNGTYDHDIYRDEAINNRFQIQ

SEQ ID NO: 5 - protein, 151 aa, Alphainfluenzavirus influenzae
YHHSNEQGSGYAADKESTQKAIDGVTNKVNSIIDKMNTQFEAVGREFNNLERRIENLNKKMEDGFLDVWTYNAELLVLMENERTLDFHDSNVKNLYDKVRLQLRDNAKELGNGCFEFYHKCDNECMESVRNGTYDYPQYSEEARLKREEIS

SEQ ID NO: 6 - protein, 151 aa, Alphainfluenzavirus influenzae
YHHENSQGSGYAADRESTQKAIDGITTKVNSIIDKMNTQFEAVGHEFSNLERRIDNLNKRMEDGFLDVWTYNAELLVLLENERTLDLHDANVKNLHERVKSQLRDNANDLGNGCFEFWHKCDNECMESVKNGTYNYPKYQAESRLNKQKIE

SEQ ID NO: 7 - protein, 151 aa, Alphainfluenzavirus influenzae
FRHQNAQGEGTAADYKSTQSAIDQITGKLNRLIEKTNQQFELIDNEFNEVEKQIGNVINWTRDSITEVWSYNAELLVAMENQHTIDLADSEMDKLYERVKRQLRENAEEDGTGCFEIFHKCDDDCMASIRNNTYDHSKYREEAMQNRIQID

SEQ ID NO: 8 - protein, 151 aa, Alphainfluenzavirus influenzae
FHHSNSEGTGMAADQKSTQEAIDKITNKVNNIVDKMNREFEVVNHEFSEVEKRINMINGKIDDQIEDLWAYNAELLVLLENQKTLDEHDSNVKNLFDEVRRRLSANAIDTGNGCFDILHKCDNECMETIKNGTYNHKEYEEEAKLERSKIN

SEQ ID NO: 9 - protein, 151 aa, Alphainfluenzavirus influenzae
FQHSNDQGVGMAADRESTQEAVDKITSKVNNIIDKMNKQYEIIDHEFSEIEARLNMINNKIDDQIQDIWAYNAELLVLLENQKTLDEHDANVNNLYNKVKRALGSNAREDGNGCFELYHKCDDQCMETIRNGTYDRQKYQEESKLERQKIE

SEQ ID NO: 10 - protein, 151 aa, Alphainfluenzavirus influenzae
FRHQNAQGTGQAADYKSTQAAIDQITGKLNRLIEKTNTEFESIESEFSEIEHQIGNIINWTKDSITDIWTYQAELLVAMENQHTIDMADSEMLNLYERVRKQLRQNAEEDGKGCFEIYHACDDSCMESIRNNTYDHSQYREEALLNRLNIN

SEQ ID NO: 11 - protein, 151 aa, Alphainfluenzavirus influenzae
FQHRNEEGTGIAADKESTQKAIDQITSKVNNIVDRMNTNFESAQHEFSEIEERINQLSKHVDDSVIDIWSYNAQLLVLLENEKTLDLHDSNVRNLHERVRRMLKDNAKDEGNGCFTFYHKCDNECIEKVRNGTYDHKEFEEESKLNRQEIE

SEQ ID NO: 12 - protein, 151 aa, Alphainfluenzavirus influenzae
FQHQNAEGTGIAADRDSTQKAIDNMQNKLNNVIDKMNKQFEVVNHEFSEVESRINMINSKIDDQITDIWAYNAELLVLLENQKTLDEHDANVRNLHDRVRRVLRENAIDTGDGCFEILHKCDNNCMDTIRNGTYNHKEYEEESKIERQKIN

SEQ ID NO: 13 - protein, 151 aa, Alphainfluenzavirus influenzae
FQHQNEQGTGIAADKESTQKAIDQITTKINNIIDKMNGNYDSIRGEFNQVEKRINMLADRIDDAVTDIWSYNAKLLVLLENDKTLDMHDANVRNLHEQVRRELKDNAIDEGNGCFELLHKCNDSCMETIRNGTYDHTEYAEESKLKRQEIN

SEQ ID NO: 14 - protein, 151 aa, Alphainfluenzavirus influenzae
FRHQNAEGTGTAADLKSTQAAIDQINGKLNRLVEKTNEKYHQIEKEFEQVEGRIQDLEKYVEDTKIDLWSYNAELLVALENQHTIDVTDSEMNKLFERVRRQLRENAEDQGNGCFEIFHQCDNNCIESIRNGTYDHNIYRDEAINNRIKIN

SEQ ID NO: 15 - protein, 151 aa, Alphainfluenzavirus influenzae
FRHQNAQGQGTAADYKSTQAAIDQITGKLNRLIEKTNQQFELIDNEFTEVEQQIGNVINWTRDSLTEIWSYNAELLVAMENQHTIDLADSEMNKLYERVRRQLRENAEEDGTGCFEIFHRCDDQCMESIRNNTYNHTEYRQESLQNRIMID

SEQ ID NO: 16 - protein, 151 aa, Alphainfluenzavirus influenzae
FQHQNEQGTGIAADKASTQKAIDEITTKINNIIEKMNGNYDSIRGEFNQVEKRINMLADRVDDAVTDVWSYNAKLLVLLENGRTLDLHDANVRNLHDQVKRALKNNAIDEGDGCFNLLHKCNDSCMETIRNGTYNHEDYQEESQLKRQEIE

SEQ ID NO: 17 - protein, 151 aa, Alphainfluenzavirus influenzae
YHHENQEGSGYAADKEATQKAVDGITNKVNSIIDKMNSQFESNIKEFNRLELRIQHLSDRVDDALLDIWSYNTELLVLLENERTLDFHDANVKNLFEKVKAQLKDNAIDEGNGCFLLLHKCNNSCMDDIKNGTYKYMDYREESHIEKQKID

SEQ ID NO: 18 - protein, 151 aa, Alphainfluenzavirus influenzae
YHHQNSEGSGYAADKEATQKAVDAITTKVNNIIDKMNTQFESTAKEFNKIEMRIKHLSDRVDDGFLDVWSYNAELLVLLENERTLDFHDANVNNLYQKVKVQLKDNAIDMGNGCFKILHKCNNTCMDDIKNGTYNYYEYRKESHLEKQKID

SEQ ID NO: 19 - protein, 55 aa, Alphainfluenzavirus influenzae
RIENLNKKVDDGFLDIWTYNAELLVLLENERTLDYHDSNVKNLYEKVRSQLKNNA

SEQ ID NO: 20 - protein, 55 aa, Alphainfluenzavirus influenzae
RLENLNKKMEDGFLDVWTYNAELLVLMENERTLDFHDSNVKNLYDKVRMQLRDNV

SEQ ID NO: 21 - protein, 55 aa, Alphainfluenzavirus influenzae
RIQDLEKYVEDTKIDLWSYNAELLVALENQHTIDLTDSEMNKLFEKTRRQLRENA

SEQ ID NO: 22 - protein, 55 aa, Alphainfluenzavirus influenzae
RIQDLEKYVEDTKIDLWSYNAEFLVALENQHTIDVTDSEMNKLFERVRRQLRENA

SEQ ID NO: 23 - protein, 55 aa, Alphainfluenzavirus influenzae
RIENLNKKMEDGFLDVWTYNAELLVLMENERTLDFHDSNVKNLYDKVRLQLRDNA

SEQ ID NO: 24 - protein, 55 aa, Alphainfluenzavirus influenzae
RIDNLNKRMEDGFLDVWTYNAELLVLLENERTLDLHDANVKNLHERVKSQLRDNA

SEQ ID NO: 25 - protein, 55 aa, Alphainfluenzavirus influenzae
QIGNVINWTRDSITEVWSYNAELLVAMENQHTIDLADSEMDKLYERVKRQLRENA

SEQ ID NO: 26 - protein, 55 aa, Alphainfluenzavirus influenzae
RINMINGKIDDQIEDLWAYNAELLVLLENQKTLDEHDSNVKNLFDEVRRRLSANA

SEQ ID NO: 27 - protein, 55 aa, Alphainfluenzavirus influenzae
RLNMINNKIDDQIQDIWAYNAELLVLLENQKTLDEHDANVNNLYNKVKRALGSNA

SEQ ID NO: 28 - protein, 55 aa, Alphainfluenzavirus influenzae
QIGNIINWTKDSITDIWTYQAELLVAMENQHTIDMADSEMLNLYERVRKQLRQNA

SEQ ID NO: 29 - protein, 55 aa, Alphainfluenzavirus influenzae
RINQLSKHVDDSVIDIWSYNAQLLVLLENEKTLDLHDSNVRNLHERVRRMLKDNA

SEQ ID NO: 30 - protein, 55 aa, Alphainfluenzavirus influenzae
RINMINSKIDDQITDIWAYNAELLVLLENQKTLDEHDANVRNLHDRVRRVLRENA

SEQ ID NO: 31 - protein, 55 aa, Alphainfluenzavirus influenzae
RINMLADRIDDAVTDIWSYNAKLLVLLENDKTLDMHDANVRNLHEQVRRELKDNA

SEQ ID NO: 32 - protein, 55 aa, Alphainfluenzavirus influenzae
RIQDLEKYVEDTKIDLWSYNAELLVALENQHTIDVTDSEMNKLFERVRRQLRENA

SEQ ID NO: 33 - protein, 55 aa, Alphainfluenzavirus influenzae
QIGNVINWTRDSLTEIWSYNAELLVAMENQHTIDLADSEMNKLYERVRRQLRENA

SEQ ID NO: 34 - protein, 55 aa, Alphainfluenzavirus influenzae
RINMLADRVDDAVTDVWSYNAKLLVLLENGRTLDLHDANVRNLHDQVKRALKNNA

SEQ ID NO: 35 - protein, 55 aa, Alphainfluenzavirus influenzae
RIQHLSDRVDDALLDIWSYNTELLVLLENERTLDFHDANVKNLFEKVKAQLKDNA

SEQ ID NO: 36 - protein, 55 aa, Alphainfluenzavirus influenzae
RIKHLSDRVDDGFLDVWSYNAELLVLLENERTLDFHDANVNNLYQKVKVQLKDNA

SEQ ID NO: 37 - protein, 55 aa, Alphainfluenzavirus influenzae
RIQDLEKYVEDTKIDLWSYNAELLVALENQHTIDLTDSEMNKLFEKTKKQLRENA

SEQ ID NO: 38 - protein, 55 aa, Alphainfluenzavirus influenzae
RVQDLEKYVEDTKIDLWSYNAELLVALENQHTIDLTDSEMNKLFEKTKKQLRENA

SEQ ID NO: 39 - protein, 9 aa, Mus musculus
GYSITSDYA

SEQ ID NO: 40 - protein, 7 aa, Mus musculus
ISYSGST

SEQ ID NO: 41 - protein, 16 aa, Mus musculus
TKNLIYYYGRPYYFDY

SEQ ID NO: 42 - protein, 6 aa, Mus musculus
QGISNY

SEQ ID NO: 43 - skipped

SEQ ID NO: 44 - protein, 9 aa, Mus musculus
QQYSKLPFT

SEQ ID NO: 45 - protein, 123 aa, Mus musculus
EVQLQESGPGLVKPSQSLSLTCTVTGYSITSDYAWNWIRQFPGNKLEWMGYISYSGSTSYNPSLKSRISITRDTSKNQFFLQLNSVTTEDTATYYCTKNLIYYYGRPYYFDYWGQGTTLTVSS

SEQ ID NO: 46 - protein, 107 aa, Mus musculus
DIQMTQTTSSLSASLGDRVTITCSASQGISNYLGWYQQKPDGTVKLLIYYTSNLHSGVPSRFSGSGSGTDYSLTISNLEPEDIATYYCQQYSKLPFTFGSGTKLEIK

SEQ ID NO: 47 - protein, 8 aa, Mus musculus
GYKFSSYW

SEQ ID NO: 48 - protein, 8 aa, Mus musculus
ILPGSGST

SEQ ID NO: 49 - protein, 8 aa, Mus musculus
ARSNWEAY

SEQ ID NO: 50 - protein, 11 aa, Mus musculus
QSLVHSNGNTY

SEQ ID NO: 51 - skipped

SEQ ID NO: 52 - protein, 9 aa, Mus musculus
SQSTHVPPT

SEQ ID NO: 53 - protein, 115 aa, Mus musculus
EVQLQQSGAELMKPGASVKISCKATGYKFSSYWIEWVKQRPGHGLEWIGKILPGSGSTNYNEKLKGKATFTADTSSNTAYMQLSSLTSEDSAVYYCARSNWEAYWGQGTLVTVSA

SEQ ID NO: 54 - protein, 112 aa, Mus musculus
DVVMTQTPLSLPVSLGDQASISCRSSQSLVHSNGNTYLHWYLQKPGQSPKLLIYKVSNRFSGVPDRFSGSGSGTDFTLKISRVEAEDLGVYFCSQSTHVPPTFGGGTKLEIK

SEQ ID NO: 55 - protein, 8 aa, Mus musculus
GYTFTSYW

SEQ ID NO: 56 - protein, 8 aa, Mus musculus
IYPSNGRT

SEQ ID NO: 57 - protein, 9 aa, Mus musculus
TIHRYDFDH

SEQ ID NO: 58 - protein, 6 aa, Mus musculus
QGINNY

SEQ ID NO: 59 - skipped

SEQ ID NO: 60 - protein, 9 aa, Mus musculus
QQYSKLPHT

SEQ ID NO: 61 - protein, 116 aa, Mus musculus
QVQLQQSGTELVKPGASVKLSCKASGYTFTSYWIHWVKQRPGQGLEWIGEIYPSNGRTNYNEKFMSKATLTVDKSSSTAYMQLSSLTSEDSAVYYCTIHRYDFDHWGQGTTLTVSS

SEQ ID NO: 62 - protein, 107 aa, Mus musculus
DIEMTQTTSSLSASLGDRVTISCSASQGINNYLNWYQQKPDGTVKLLIYYTSSLHSGVPSRFSGSGSGTDYSLTISILEPEDIATYYCQQYSKLPHTFGGGTKLEIK

SEQ ID NO: 63 - protein, 8 aa, Mus musculus
GFTFSRYY

SEQ ID NO: 64 - protein, 8 aa, Mus musculus
INNNGGST

SEQ ID NO: 65 - protein, 9 aa, Mus musculus
TSHGPWFTY

SEQ ID NO: 66 - protein, 6 aa, Mus musculus
QDINSH

SEQ ID NO: 67 - skipped

SEQ ID NO: 68 - protein, 9 aa, Mus musculus
LQYDEFPPT

SEQ ID NO: 69 - protein, 116 aa, Mus musculus
EVQLVESGGGLVKLGGSLKLSCAASGFTFSRYYMSWVRQTPEKRLELVAAINNNGGSTYYPDTVKGRFTISRDNAKNTLYLQMSSLKSEDTALYYCTSHGPWFTYWGQGTLVTVSA

SEQ ID NO: 70 - protein, 107 aa, Mus musculus
DIKMTQSPSSMYASLGERVTITCKASQDINSHLSWFQQKPGKSPKTLIYRANRLVDGVPSRFSGSGSGQDYSLTISSLEYEDLGIYYCLQYDEFPPTFGGGTKLEIK

SEQ ID NO: 71 - protein, 8 aa, Homo sapiens
GVSMNSNH

SEQ ID NO: 72 - protein, 7 aa, Homo sapiens
IYYTGKT

SEQ ID NO: 73 - protein, 18 aa, Homo sapiens
ARRAMASVQRGILRVFDL

SEQ ID NO: 74 - protein, 6 aa, Homo sapiens
QIIDKW

SEQ ID NO: 75 - skipped

SEQ ID NO: 76 - protein, 10 aa, Homo sapiens
QQYKSYLPYT

SEQ ID NO: 77 - protein, 124 aa, Homo sapiens
QVQLQESGPGLVKPSETLSLTCTVSGVSMNSNHWSWIRQAPGKELEWIGYIYYTGKTFYNPSLQSRVTVSLDTSKNQFYLKLTSVTAADTAVYYCARRAMASVQRGILRVFDLWGQGKMVTVSS

SEQ ID NO: 78 - protein, 108 aa, Homo sapiens
DIQMTQSPSTLSASVGDRVTITCRASQIIDKWLAWYQHKPGKAPKLLIYEASNLETGVPSRFSGSGSGTEFTLTISSLQPDDFATYFCQQYKSYLPYTFGQGTKLEIK

SEQ ID NO: 79 - protein, 8 aa, Homo sapiens
GPMFSRSA

SEQ ID NO: 80 - protein, 8 aa, Homo sapiens
IIPTVDLK

SEQ ID NO: 81 - protein, 14 aa, Homo sapiens
ARMGSGSSYYGMDV

SEQ ID NO: 82 - protein, 11 aa, Homo sapiens
QSLLQSNGNNY

SEQ ID NO: 83 - skipped

SEQ ID NO: 84 - protein, 10 aa, Homo sapiens
LQARQSSVLT

SEQ ID NO: 85 - protein, 121 aa, Homo sapiens
QVQLEQSGAEVKKPGSSVKVSCKASGPMFSRSAFSWVRQAPGQGLEWMGRIIPTVDLKNYAQKFQGRVTFTADKSTATSYMELRSLKSEDTAVYYCARMGSGSSYYGMDVWGLGTTVTVSS

SEQ ID NO: 86 - protein, 113 aa, Homo sapiens
DIVMTQSPLSLPVIPGEPASISCRSSQSLLQSNGNNYLDWYLQKPGQSPQLLIYLGSNRASGVPDRFSGSGSGTDFTLTISRVEAEDVGVYYCLQARQSSVLTFGGGTKLEIK

SEQ ID NO: 87 - protein, 10 aa, Homo sapiens
GGPLTSSTYF

SEQ ID NO: 88 - protein, 7 aa, Homo sapiens
INFRGTT

SEQ ID NO: 89 - protein, 18 aa, Homo sapiens
ARHTQRLTVFTVVHGFDL

SEQ ID NO: 90 - protein, 9 aa, Homo sapiens
TGDIGVSDF

SEQ ID NO: 91 - skipped

SEQ ID NO: 92 - protein, 11 aa, Homo sapiens
CLYSTRSRDWE

SEQ ID NO: 93 - protein, 126 aa, Homo sapiens
QVQLQESGPGLVKPSETLSLTCSVSGGPLTSSTYFWGWIRQPPGKGLEWLGSINFRGTTDNAPSLKSRVTLSIDTSTHQFSLRLSSVTAKDTAVYYCARHTQRLTVFTVVHGFDLWGQGTVVSVSS

SEQ ID NO: 94 - protein, 111 aa, Homo sapiens
QSALTQPASVSGSPGQSITISCTGATGDIGVSDFVSWYQQHPGKAPKLIIFDVTNRPSGVSNRFSGSKSVNTASLTISGLQAEDEADYYCCLYSTRSRDWEFGGGTKLTVL

SEQ ID NO: 95 - protein, 55 aa, Alphainfluenzavirus influenzae; identical to SEQ ID NO: 37

SEQ ID NO: 96 - protein, 55 aa, Alphainfluenzavirus influenzae
RMENLNKKVDDGFLDIWTYNAELLVLLENERTLDFHDSNVKNLYEKVKSQLKNNA

SEQ ID NO: 97 - protein, 55 aa, Alphainfluenzavirus influenzae
RIENLNKKVDDGFLDIWTYNAELLVLLENERTLDYHDSNVKNLYEKVRNQLKNNA

SEQ ID NO: 98 - protein, 55 aa, Alphainfluenzavirus influenzae; identical to SEQ ID NO: 97